European Patent Application EP 4 714 453 A1, published March 25, 2026. Title: 核酸送達用構造体の造血器腫瘍の治療への使用. Applicant: 国立研究開発法人科学技術振興機構. The sequence listing filed with the application follows.

SEQUENCE LISTING (32 sequences)

SEQ ID NO: 1 - RNA, 24 nt, synthetic construct
  source 1..24: mol_type = other RNA
tgaggtgcagtgctgcatctctgg

SEQ ID NO: 2 - RNA, 24 nt, synthetic construct
  source 1..24: mol_type = other RNA
  misc_feature 1..2: note = Linked to the 3' side nucleoside by -P(S)OH-.
  misc_feature 1..24: note = The 1,6,8,11,13,14,16,18,19,20,21,22nd nucleotides are 2'-F RNAs.
tgaggtgcagtgctgcatctctgg

SEQ ID NO: 3 - RNA, 24 nt, synthetic construct
  source 1..24: mol_type = other RNA
  misc_feature 1..2: note = Linked to the 3' side nucleoside by -P(S)OH-.
  misc_feature 1..24: note = The 1,6,8,11,13,14,16,18,19,20,21,22nd nucleotides are 2'-OMe RNAs.
tgaggtgcagtgctgcatctctgg

SEQ ID NO: 4 - RNA, 24 nt, synthetic construct
  source 1..24: mol_type = other RNA
  misc_feature 1..2: note = Linked to the 3' side nucleoside by -P(S)OH-.
  misc_feature 1..24: note = The 1,6,8,11,13,14,16,18,19,20,21,22nd nucleotides are 2'-F RNAs.
tgaggtgcagtgctgcatctctgg

SEQ ID NO: 5 - RNA, 22 nt, synthetic construct
  source 1..22: mol_type = other RNA
  misc_feature 22: note = ^dT^dT is linked to the 3' end.
  misc_feature 1..2: note = Linked to the 3' side nucleoside by -P(S)OH-.
  misc_feature 1..22: note = The odd-numbered nucleotides are 2'-F RNAs and the rest nucleotides are 2'-OMe RNAs.
tgagatgaagcactgtagctca

SEQ ID NO: 6 - RNA, 22 nt, synthetic construct
  source 1..22: mol_type = other RNA
  misc_feature 22: note = ^dT^dT is linked to the 3' end.
  misc_feature 1: note = -P(O)(OH)2 is linked to the 5' end.
  misc_feature 1..22: note = The odd-numbered nucleotides are 2'-F RNAs and the rest nucleotides are 2'-OMe RNAs.
  misc_feature 1..2: note = Linked to the 3' side nucleoside by -P(S)OH-.
tgagatgaagcactgtagctca

SEQ ID NO: 7 - RNA, 22 nt, synthetic construct
  source 1..22: mol_type = other RNA
  misc_feature 22: note = ^dT^dT is linked to the 3' end.
  misc_feature 1..2: note = Linked to the 3' side nucleoside by -P(S)OH-.
  misc_feature 1..22: note = The 1,2,3,7,8,9,13,14,15,19,20,21,22nd nucleotides are 2'-OMe RNAs.
tgagatgaagcactgtagctca

SEQ ID NO: 8 - RNA, 22 nt, synthetic construct
  source 1..22: mol_type = other RNA
  misc_feature 22: note = ^dT^dT is linked to the 3' end.
  misc_feature 1..2: note = Linked to the 3' side nucleoside by -P(S)OH-.
  misc_feature 1..22: note = he 1,2,3,7,8,9,13,14,15,19,20,21,22nd nucleotides are 2'-F RNAs and the rest nucleotides are 2'-OMe RNAs.
tgagatgaagcactgtagctca

SEQ ID NO: 9 - RNA, 22 nt, synthetic construct
  source 1..22: mol_type = other RNA
  misc_feature 22: note = ^dT^dT is linked to the 3' end.
  misc_feature 1..2: note = Linked to the 3' side nucleoside by -P(S)OH-.
  misc_feature 1..22: note = The 1,6,11,13,14,16,19,20,21nd nucleotides are 2'-F RNAs.
tgagatgaagcactgtagctca

SEQ ID NO: 10 - RNA, 22 nt, synthetic construct
  source 1..22: mol_type = other RNA
  misc_feature 22: note = ^dG^dG is linked to the 3' end.
  misc_feature 1..2: note = Linked to the 3' side nucleoside by -P(S)OH-.
  misc_feature 1..22: note = The odd-numbered nucleotides are 2'-F RNAs and the rest nucleotides are 2'-OMe RNAs.
tgagatgaagcactgtagctca

SEQ ID NO: 11 - RNA, 22 nt, synthetic construct
  source 1..22: mol_type = other RNA
  misc_feature 22: note = ^Gm^Gm is linked to the 3' end.
  misc_feature 1..2: note = Linked to the 3' side nucleoside by -P(S)OH-.
  misc_feature 1..22: note = The odd-numbered nucleotides are 2'-F RNAs and the rest nucleotides are 2'-OMe RNAs.
tgagatgaagcactgtagctca

SEQ ID NO: 12 - RNA, 22 nt, synthetic construct
  source 1..22: mol_type = other RNA
  misc_feature 22: note = ^Gf^Gf is linked to the 3' end.
  misc_feature 1..2: note = Linked to the 3' side nucleoside by -P(S)OH-.
  misc_feature 1..22: note = The odd-numbered nucleotides are 2'-F RNAs and the rest nucleotides are 2'-OMe RNAs.
tgagatgaagcactgtagctca

SEQ ID NO: 13 - RNA, 22 nt, synthetic construct
  source 1..22: mol_type = other RNA
  misc_feature 22: note = ^dT^dT is linked to the 3' end.
  misc_feature 1: note = VP- is linked to the 5' end.
  misc_feature 1..2: note = Linked to the 3' side nucleoside by -P(S)OH-.
  misc_feature 1..22: note = The 3,5,7,9,11,13,15,17,19,21nd nucleotides are 2'-F RNAs and the rest nucleotides are 2'-OMe RNAs.
tgagatgaagcactgtagctca

SEQ ID NO: 14 - RNA, 22 nt, synthetic construct
  source 1..22: mol_type = other RNA
  misc_feature 22: note = ^dT^dT is linked to the 3' end.
  misc_feature 1..2: note = Linked to the 3' side nucleoside by -P(S)OH-.
  misc_feature 1..22: note = The odd-numbered nucleotides are 2'-F RNAs and the rest nucleotides are 2'-OMe RNAs.
tgagatgaagcactgtagctaa

SEQ ID NO: 15 - RNA, 22 nt, synthetic construct
  source 1..22: mol_type = other RNA
  misc_feature 22: note = ^dG^dG is linked to the 3' end.
  misc_feature 1: note = -P(O)(OH)2 is linked to the 5' end.
tgagatgaagcactgtagctca

SEQ ID NO: 16 - RNA, 22 nt, synthetic construct
  source 1..22: mol_type = other RNA
  misc_feature 22: note = ^Gm^Gm is linked to the 3' end.
  misc_feature 1: note = -P(O)(OH)2 is linked to the 5' end.
tgagatgaagcactgtagctca

SEQ ID NO: 17 - RNA, 22 nt, synthetic construct
  source 1..22: mol_type = other RNA
  misc_feature 22: note = ^Gf^Gf is linked to the 3' end.
  misc_feature 1: note = -P(O)(OH)2 is linked to the 5' end.
tgagatgaagcactgtagctca

SEQ ID NO: 18 - RNA, 22 nt, synthetic construct
  source 1..22: mol_type = other RNA
  misc_feature 22: note = ^dT^dT is linked to the 3' end.
  misc_feature 1: note = -P(O)(OH)2 is linked to the 5' end.
tgagatgaagcactgtagctca

SEQ ID NO: 19 - RNA, 22 nt, synthetic construct
  source 1..22: mol_type = other RNA
  misc_feature 22: note = ^dT^dT is linked to the 3' end.
  misc_feature 1: note = -P(O)(OH)2 is linked to the 5' end.
tgagatgaagcactgtagctaa

SEQ ID NO: 20 - RNA, 22 nt, synthetic construct
  source 1..22: mol_type = other RNA
  misc_feature 22: note = Am^Am is linked to the 3' end.
  misc_feature 1: note = -P(O)(OH)2 is linked to the 5' end.
tgagatgaagcactgtagctca

SEQ ID NO: 21 - RNA, 22 nt, synthetic construct
  source 1..22: mol_type = other RNA
tgagctacagtgctgcatctct

SEQ ID NO: 22 - RNA, 22 nt, synthetic construct
  source 1..22: mol_type = other RNA
  misc_feature 22: note = *X*X*X*X*X*X*Y*Z is linked to the 3' end.
  misc_feature 1..22: note = Linked to the 3' side nucleoside by -P(S)OH-.
tgagctacagtgctgcatctct

SEQ ID NO: 23 - RNA, 22 nt, synthetic construct
  source 1..22: mol_type = other RNA
  misc_feature 22: note = *X*X*X*X*X*X*Y*Glu is linked to the 3' end.
  misc_feature 1..22: note = Linked to the 3' side nucleoside side by cationic backbone.
tgagctacagtgctgcatctct

SEQ ID NO: 24 - RNA, 19 nt, synthetic construct
  source 1..19: mol_type = other RNA
  misc_feature 19: note = ^dT^dT is linked to the 3' end.
ggcctttcactactcctac

SEQ ID NO: 25 - RNA, 19 nt, synthetic construct
  source 1..19: mol_type = other RNA
  misc_feature 19: note = ^t^t*X*X*X*X*X*X*Y*Z is linked to the 3' end.
  misc_feature 1..19: note = Linked to the 3' side nucleoside by -P(S)OH-.
gtaggagtagtgaaaggcc

SEQ ID NO: 26 - RNA, 19 nt, synthetic construct
  source 1..19: mol_type = other RNA
  misc_feature 19: note = ^t^t*X*X*X*X*X*X*Y*Glu is linked to the 3' end.
  misc_feature 1..19: note = Linked to the 3' side nucleoside side by cationic backbone.
gtaggagtagtgaaaggcc

SEQ ID NO: 27 - DNA, 20 bp, synthetic construct
  source 1..20: mol_type = other DNA
cctcctcacttggctgtctg

SEQ ID NO: 28 - DNA, 20 bp, synthetic construct
  source 1..20: mol_type = other DNA
tcacgtttgcggtttggttc

SEQ ID NO: 29 - DNA, 20 bp, synthetic construct
  source 1..20: mol_type = other DNA
tggtggtgtgccaagacatt

SEQ ID NO: 30 - DNA, 20 bp, synthetic construct
  source 1..20: mol_type = other DNA
cacctcaccatgccatctca

SEQ ID NO: 31 - DNA, 24 bp, synthetic construct
  source 1..24: mol_type = other DNA
tctagacggcaggtcaggtccacc

SEQ ID NO: 32 - DNA, 24 bp, synthetic construct
  source 1..24: mol_type = other DNA
ccacccatggcaaattccatggca